European Patent Application EP 4 212 547 A1, published July 19, 2023. Title: MODIFIED CHIMERIC RECEPTORS AND RELATED COMPOSITIONS AND METHODS. Applicant: Juno Therapeutics, Inc. Application EP. The sequence listing filed with the application follows.

SEQUENCE LISTING (184 sequences)

SEQ ID NO: 1 - protein, 12 aa, synthetic construct
  REGION 1..12: note = IgG4 hinge
ESKYGPPCPPCP

SEQ ID NO: 2 - protein, 27 aa, synthetic construct
  REGION 1..27: note = CD28 transmembrane domain
FWVLVVVGGVLACYSLLVTVAFIIFWV

SEQ ID NO: 3 - protein, 42 aa, Homo sapiens
  REGION 1..42: note = 4-1BB costimulatory domain
KRGRKKLLYIFKQPFMRPVQTTQEEDGCSCRFPEEEEGGCEL

SEQ ID NO: 4 - protein, 112 aa, synthetic construct
  REGION 1..112: note = CD3-zeta intracellular signaling domain
RVKFSRSADAPAYQQGQNQLYNELNLGRREEYDVLDKRRGRDPEMGGKPRRKNPQEGLYNELQKDKMAEAYSEIGMKGERRRGKGHDGLYQGLSTATKDTYDALHMQALPPR

SEQ ID NO: 5 - protein, 69 aa, synthetic construct
  REGION 1..69: note = CD28-4-1BB
FWVLVVVGGVLACYSLLVTVAFIIFWVKRGRKKLLYIFKQPFMRPVQTTQEEDGCSCRFPEEEEGGCEL

SEQ ID NO: 6 - protein, 30 aa, synthetic construct
CYSLLVTVAFIIFWVKRGRKKLLYIFKQPF

SEQ ID NO: 7 - protein, 16 aa, synthetic construct
VAFIIFWVKRGRKKLL

SEQ ID NO: 8 - protein, 15 aa, synthetic construct
AFIIFWVKRGRKKLL

SEQ ID NO: 9 - protein, 15 aa, synthetic construct
FWVKRGRKKLLYIFK

SEQ ID NO: 10 - protein, 14 aa, synthetic construct
FIIFWVKRGRKKLL

SEQ ID NO: 11 - protein, 13 aa, synthetic construct
FIIFWVKRGRKKL

SEQ ID NO: 12 - protein, 13 aa, synthetic construct
IIFWVKRGRKKLL

SEQ ID NO: 13 - protein, 32 aa, synthetic construct
  REGION 1..32: note = Variant junction region
CYSLLVTVAFIIFWVNNKRGRKKLLYIFKQPF

SEQ ID NO: 14 - protein, 14 aa, synthetic construct
  REGION 1..14: note = Variant peptide
IIFWVNNKRGRKKL

SEQ ID NO: 15 - protein, 13 aa, synthetic construct
  REGION 1..13: note = Variant peptide
IIFWVNNKRGRKK

SEQ ID NO: 16 - protein, 9 aa, synthetic construct
VAFIIFWVK

SEQ ID NO: 17 - protein, 9 aa, synthetic construct
AFIIFWVKR

SEQ ID NO: 18 - protein, 9 aa, synthetic construct
FIIFWVKRG

SEQ ID NO: 19 - protein, 9 aa, synthetic construct
IIFWVKRGR

SEQ ID NO: 20 - protein, 9 aa, synthetic construct
IFWVKRGRK

SEQ ID NO: 21 - protein, 9 aa, synthetic construct
FWVKRGRKK

SEQ ID NO: 22 - protein, 9 aa, synthetic construct
WVKRGRKKL

SEQ ID NO: 23 - protein, 9 aa, synthetic construct
  REGION 1..9: note = Synthetic peptide K28S
VAFIIFWVS

SEQ ID NO: 24 - protein, 9 aa, synthetic construct
  REGION 1..9: note = Synthetic peptide K28S
AFIIFWVSR

SEQ ID NO: 25 - protein, 9 aa, synthetic construct
  REGION 1..9: note = Synthetic peptide K28S
FIIFWVSRG

SEQ ID NO: 26 - protein, 9 aa, synthetic construct
  REGION 1..9: note = Synthetic peptide K28S
IIFWVSRGR

SEQ ID NO: 27 - protein, 9 aa, synthetic construct
  REGION 1..9: note = Synthetic peptide K28S
IFWVSRGRK

SEQ ID NO: 28 - protein, 9 aa, synthetic construct
  REGION 1..9: note = Synthetic peptide K28S
FWVSRGRKK

SEQ ID NO: 29 - protein, 9 aa, synthetic construct
  REGION 1..9: note = Synthetic peptide K28S
WVSRGRKKL

SEQ ID NO: 30 - protein, 9 aa, synthetic construct
  REGION 1..9: note = Synthetic peptide K28L
VAFIIFWVL

SEQ ID NO: 31 - protein, 9 aa, synthetic construct
  REGION 1..9: note = Synthetic peptide K28L
AFIIFWVLR

SEQ ID NO: 32 - protein, 9 aa, synthetic construct
  REGION 1..9: note = Synthetic peptide K28L
FIIFWVLRG

SEQ ID NO: 33 - protein, 9 aa, synthetic construct
  REGION 1..9: note = Synthetic peptide K28L
IIFWVLRGR

SEQ ID NO: 34 - protein, 9 aa, synthetic construct
  REGION 1..9: note = Synthetic peptide K28L
IFWVLRGRK

SEQ ID NO: 35 - protein, 9 aa, synthetic construct
  REGION 1..9: note = Synthetic peptide K28L
FWVLRGRKK

SEQ ID NO: 36 - protein, 9 aa, synthetic construct
  REGION 1..9: note = Synthetic peptide K28L
WVLRGRKKL

SEQ ID NO: 37 - protein, 9 aa, synthetic construct
  REGION 1..9: note = Synthetic peptide K28H
VAFIIFWVH

SEQ ID NO: 38 - protein, 9 aa, synthetic construct
  REGION 1..9: note = Synthetic peptide K28H
AFIIFWVHR

SEQ ID NO: 39 - protein, 9 aa, synthetic construct
  REGION 1..9: note = Synthetic peptide K28H
FIIFWVHRG

SEQ ID NO: 40 - protein, 9 aa, synthetic construct
  REGION 1..9: note = Synthetic peptide K28H
IIFWVHRGR

SEQ ID NO: 41 - protein, 9 aa, synthetic construct
  REGION 1..9: note = Synthetic peptide K28H
IFWVHRGRK

SEQ ID NO: 42 - protein, 9 aa, synthetic construct
  REGION 1..9: note = Synthetic peptide K28H
FWVHRGRKK

SEQ ID NO: 43 - protein, 9 aa, synthetic construct
  REGION 1..9: note = Synthetic peptide K28H
WVHRGRKKL

SEQ ID NO: 44 - protein, 9 aa, synthetic construct
  REGION 1..9: note = Synthetic peptide K28A
VAFIIFWVA

SEQ ID NO: 45 - protein, 9 aa, synthetic construct
  REGION 1..9: note = Synthetic peptide K28A
AFIIFWVAR

SEQ ID NO: 46 - protein, 9 aa, synthetic construct
  REGION 1..9: note = Synthetic peptide K28A
IIFWVARGR

SEQ ID NO: 47 - protein, 9 aa, synthetic construct
  REGION 1..9: note = Synthetic peptide K28A
IFWVARGRK

SEQ ID NO: 48 - protein, 9 aa, synthetic construct
  REGION 1..9: note = Synthetic peptide K28A
FWVARGRKK

SEQ ID NO: 49 - protein, 9 aa, synthetic construct
  REGION 1..9: note = Synthetic peptide K28A
WVARGRKKL

SEQ ID NO: 50 - protein, 9 aa, synthetic construct
  REGION 1..9: note = Synthetic peptide K28Q
VAFIIFWVQ

SEQ ID NO: 51 - protein, 9 aa, synthetic construct
  REGION 1..9: note = Synthetic peptide K28Q
AFIIFWVQR

SEQ ID NO: 52 - protein, 9 aa, synthetic construct
  REGION 1..9: note = Synthetic peptide K28Q
FIIFWVQRG

SEQ ID NO: 53 - protein, 9 aa, synthetic construct
  REGION 1..9: note = Synthetic peptide K28Q
IIFWVQRGR

SEQ ID NO: 54 - protein, 9 aa, synthetic construct
  REGION 1..9: note = Synthetic peptide K28Q
IFWVQRGRK

SEQ ID NO: 55 - protein, 9 aa, synthetic construct
  REGION 1..9: note = Synthetic peptide K28Q
FWVQRGRKK

SEQ ID NO: 56 - protein, 9 aa, synthetic construct
  REGION 1..9: note = Synthetic peptide K28Q
WVQRGRKKL

SEQ ID NO: 57 - protein, 9 aa, synthetic construct
  REGION 1..9: note = Synthetic peptide R31S
IIFWVKRGS

SEQ ID NO: 58 - protein, 9 aa, synthetic construct
  REGION 1..9: note = Synthetic peptide R31S
IFWVKRGSK

SEQ ID NO: 59 - protein, 9 aa, synthetic construct
  REGION 1..9: note = Synthetic peptide R31S
FWVKRGSKK

SEQ ID NO: 60 - protein, 9 aa, synthetic construct
  REGION 1..9: note = Synthetic peptide R31S
WVKRGSKKL

SEQ ID NO: 61 - protein, 9 aa, synthetic construct
  REGION 1..9: note = Synthetic peptide R31L
IIFWVKRGL

SEQ ID NO: 62 - protein, 9 aa, synthetic construct
  REGION 1..9: note = Synthetic peptide R31L
IFWVKRGLK

SEQ ID NO: 63 - protein, 9 aa, synthetic construct
  REGION 1..9: note = Synthetic peptide R31L
FWVKRGLKK

SEQ ID NO: 64 - protein, 9 aa, synthetic construct
  REGION 1..9: note = Synthetic peptide R31L
WVKRGLKKL

SEQ ID NO: 65 - protein, 9 aa, synthetic construct
  REGION 1..9: note = Synthetic peptide R31H
IIFWVKRGH

SEQ ID NO: 66 - protein, 9 aa, synthetic construct
  REGION 1..9: note = Synthetic peptide R31H
IFWVKRGHK

SEQ ID NO: 67 - protein, 9 aa, synthetic construct
  REGION 1..9: note = Synthetic peptide R31H
FWVKRGHKK

SEQ ID NO: 68 - protein, 9 aa, synthetic construct
  REGION 1..9: note = Synthetic peptide R31H
WVKRGHKKL

SEQ ID NO: 69 - protein, 9 aa, synthetic construct
  REGION 1..9: note = Synthetic peptide R31A
IIFWVKRGA

SEQ ID NO: 70 - protein, 9 aa, synthetic construct
  REGION 1..9: note = Synthetic peptide R31A
IFWVKRGAK

SEQ ID NO: 71 - protein, 9 aa, synthetic construct
  REGION 1..9: note = Synthetic peptide R31A
FWVKRGAKK

SEQ ID NO: 72 - protein, 9 aa, synthetic construct
  REGION 1..9: note = Synthetic peptide R31A
WVKRGAKKL

SEQ ID NO: 73 - protein, 9 aa, synthetic construct
  REGION 1..9: note = Synthetic peptide R31N
IIFWVKRGN

SEQ ID NO: 74 - protein, 9 aa, synthetic construct
  REGION 1..9: note = Synthetic peptide R31N
IFWVKRGNK

SEQ ID NO: 75 - protein, 9 aa, synthetic construct
  REGION 1..9: note = Synthetic peptide R31N
FWVKRGNKK

SEQ ID NO: 76 - protein, 9 aa, synthetic construct
  REGION 1..9: note = Synthetic peptide R31N
WVKRGNKKL

SEQ ID NO: 77 - protein, 9 aa, synthetic construct
  REGION 1..9: note = Synthetic peptide K28Q/R31S
IIFWVQRGS

SEQ ID NO: 78 - protein, 9 aa, synthetic construct
  REGION 1..9: note = Synthetic peptide K28Q/R31S
IFWVQRGSK

SEQ ID NO: 79 - protein, 9 aa, synthetic construct
  REGION 1..9: note = Synthetic peptide K28Q/R31S
FWVQRGSKK

SEQ ID NO: 80 - protein, 9 aa, synthetic construct
  REGION 1..9: note = Synthetic peptide K28Q/R31S
WVQRGSKKL

SEQ ID NO: 81 - protein, 9 aa, synthetic construct
  REGION 1..9: note = Synthetic peptide K28Q/R31A
IIFWVQRGA

SEQ ID NO: 82 - protein, 9 aa, synthetic construct
  REGION 1..9: note = Synthetic peptide K28Q/R31A
IFWVQRGAK

SEQ ID NO: 83 - protein, 9 aa, synthetic construct
  REGION 1..9: note = Synthetic peptide K28Q/R31A
FWVQRGAKK

SEQ ID NO: 84 - protein, 9 aa, synthetic construct
  REGION 1..9: note = Synthetic peptide K28Q/R31A
WVQRGAKKL

SEQ ID NO: 85 - protein, 9 aa, synthetic construct
  REGION 1..9: note = Synthetic peptide K28Q/R31N
IIFWVQRGN

SEQ ID NO: 86 - protein, 9 aa, synthetic construct
  REGION 1..9: note = Synthetic peptide K28Q/R31N
IFWVQRGNK

SEQ ID NO: 87 - protein, 9 aa, synthetic construct
  REGION 1..9: note = Synthetic peptide K28Q/R31N
FWVQRGNKK

SEQ ID NO: 88 - protein, 9 aa, synthetic construct
  REGION 1..9: note = Synthetic peptide K28Q/R31N
WVQRGNKKL

SEQ ID NO: 89 - protein, 9 aa, synthetic construct
  REGION 1..9: note = Synthetic peptide L34S
WVKRGRKKS

SEQ ID NO: 90 - protein, 9 aa, synthetic construct
  REGION 1..9: note = Synthetic peptide L34A
WVKRGRKKA

SEQ ID NO: 91 - protein, 9 aa, synthetic construct
  REGION 1..9: note = Synthetic peptide K28Q/L34S
WVQRGNKKS

SEQ ID NO: 92 - protein, 9 aa, synthetic construct
  REGION 1..9: note = Synthetic peptide K28Q/L34A
WVQRGNKKA

SEQ ID NO: 93 - protein, 255 aa, Homo sapiens
  REGION 1..255: note = 4-1BB
MGNSCYNIVATLLLVLNFERTRSLQDPCSNCPAGTFCDNNRNQICSPCPPNSFSSAGGQRTCDICRQCKGVFRTRKECSSTSNAECDCTPGFHCLGAGCSMCEQDCKQGQELTKKGCKDCCFGTFNDQKRGICRPWTNCSLDGKSVLVNGTKERDVVCGPSPADLSPGASSVTPPAPAREPGHSPQIISFFLALTSTALLFLLFFLTLRFSVVKRGRKKLLYIFKQPFMRPVQTTQEEDGCSCRFPEEEEGGCEL

SEQ ID NO: 94 - protein, 255 aa, Homo sapiens; identical to SEQ ID NO: 93
  REGION 1..255: note = CD28

SEQ ID NO: 95 - protein, 164 aa, Homo sapiens
  REGION 1..164: note = CD3 zeta chain
MKWKALFTAAILQAQLPITEAQSFGLLDPKLCYLLDGILFIYGVILTALFLRVKFSRSADAPAYQQGQNQLYNELNLGRREEYDVLDKRRGRDPEMGGKPQRRKNPQEGLYNELQKDKMAEAYSEIGMKGERRRGKGHDGLYQGLSTATKDTYDALHMQALPPR

SEQ ID NO: 96 - protein, 14 aa, synthetic construct
  REGION 1..14: note = Synthetic
FIIFWVNNKRGRKK

SEQ ID NO: 97 - protein, 14 aa, synthetic construct
  REGION 1..14: note = Synthetic
IFWVNNKRGRKKLL

SEQ ID NO: 98 - protein, 14 aa, synthetic construct
  REGION 1..14: note = Synthetic
FIIFWVNNKRGRKK

SEQ ID NO: 99 - protein, 14 aa, synthetic construct
  REGION 1..14: note = Synthetic
IFWVNNKRGRKKLL

SEQ ID NO: 100 - protein, 9 aa, synthetic construct
  REGION 1..9: note = Synthetic peptide K28R
VAFIIFWVR

SEQ ID NO: 101 - protein, 9 aa, synthetic construct
  REGION 1..9: note = Synthetic peptide K28R
AFIIFWVRR

SEQ ID NO: 102 - protein, 9 aa, synthetic construct
  REGION 1..9: note = Synthetic peptide K28A
FIIFWVARG

SEQ ID NO: 103 - protein, 28 aa, Homo sapiens
  REGION 1..28: note = CD28 transmembrane domain
MFWVLVVVGGVLACYSLLVTVAFIIFWV

SEQ ID NO: 104 - protein, 66 aa, Homo sapiens
  REGION 1..66: note = CD28
IEVMYPPPYLDNEKSNGTIIHVKGKHLCPSPLFPGPSKPFWVLVVVGGVLACYSLLVTVAFIIFWV

SEQ ID NO: 105 - protein, 112 aa, Homo sapiens
  REGION 1..112: note = CD3 zeta
RVKFSRSAEPPAYQQGQNQLYNELNLGRREEYDVLDKRRGRDPEMGGKPRRKNPQEGLYNELQKDKMAEAYSEIGMKGERRRGKGHDGLYQGLSTATKDTYDALHMQALPPR

SEQ ID NO: 106 - DNA, 36 bp, Homo sapiens
  misc_feature 1..36: note = spacer (IgG4hinge)
  source 1..36: mol_type = unassigned DNA
gaatctaagtacggaccgccctgccccccttgccct

SEQ ID NO: 107 - protein, 119 aa, Homo sapiens
  REGION 1..119: note = Hinge-CH3 spacer
ESKYGPPCPPCPGQPREPQVYTLPPSQEEMTKNQVSLTCLVKGFYPSDIAVEWESNGQPENNYKTTPPVLDSDGSFFLYSRLTVDKSRWQEGNVFSCSVMHEALHNHYTQKSLSLSLGK

SEQ ID NO: 108 - protein, 229 aa, Homo sapiens
  REGION 1..229: note = Hinge-CH2-CH3 spacer
ESKYGPPCPPCPAPEFLGGPSVFLFPPKPKDTLMISRTPEVTCVVVDVSQEDPEVQFNWYVDGVEVHNAKTKPREEQFNSTYRVVSVLTVLHQDWLNGKEYKCKVSNKGLPSSIEKTISKAKGQPREPQVYTLPPSQEEMTKNQVSLTCLVKGFYPSDIAVEWESNGQPENNYKTTPPVLDSDGSFFLYSRLTVDKSRWQEGNVFSCSVMHEALHNHYTQKSLSLSLGK

SEQ ID NO: 109 - protein, 282 aa, Homo sapiens
  REGION 1..282: note = IgD-hinge-Fc
RWPESPKAQASSVPTAQPQAEGSLAKATTAPATTRNTGRGGEEKKKEKEKEEQEERETKTPECPSHTQPLGVYLLTPAVQDLWLRDKATFTCFVVGSDLKDAHLTWEVAGKVPTGGVEEGLLERHSNGSQSQHSRLTLPRSLWNAGTSVTCTLNHPSLPPQRLMALREPAAQAPVKLSLNLLASSDPPEAASWLLCEVSGFSPPNILLMWLEDQREVNTSGFAPARPPPQPGSTTFWAWSVLRVPAPPSPQPATYTCVVSHEDSRTLLNASRSLEVSYVTDH

SEQ ID NO: 110 - protein, 24 aa, synthetic construct
  REGION 1..24: note = T2A
LEGGGEGRGSLLTCGDVEENPGPR

SEQ ID NO: 111 - protein, 357 aa, synthetic construct
  REGION 1..357: note = tEGFR
MLLLVTSLLLCELPHPAFLLIPRKVCNGIGIGEFKDSLSINATNIKHFKNCTSISGDLHILPVAFRGDSFTHTPPLDPQELDILKTVKEITGFLLIQAWPENRTDLHAFENLEIIRGRTKQHGQFSLAVVSLNITSLGLRSLKEISDGDVIISGNKNLCYANTINWKKLFGTSGQKTKIISNRGENSCKATGQVCHALCSPEGCWGPEPRDCVSCRNVSRGRECVDKCNLLEGEPREFVENSECIQCHPECLPQAMNITCTGRGPDNCIQCAHYIDGPHCVKTCPAGVMGENNTLVWKYADAGHVCHLCHPNCTYGCTGPGLEGCPTNGPKIPSIATGMVGALLLLLVVALGIGLFM

SEQ ID NO: 112 - protein, 41 aa, Homo sapiens
  REGION 1..41: note = CD28 cytoplasmic domain
RSKRSRLLHSDYMNMTPRRPGPTRKHYQPYAPPRDFAAYRS

SEQ ID NO: 113 - protein, 41 aa, Homo sapiens
  REGION 1..41: note = CD28 cytoplasmic domain
RSKRSRGGHSDYMNMTPRRPGPTRKHYQPYAPPRDFAAYRS

SEQ ID NO: 114 - protein, 69 aa, synthetic construct
  REGION 1..69: note = Synthetic K28A
FWVLVVVGGVLACYSLLVTVAFIIFWVARGRKKLLYIFKQPFMRPVQTTQEEDGCSCRFPEEEEGGCEL

SEQ ID NO: 115 - protein, 69 aa, synthetic construct
  REGION 1..69: note = Synthetic K28H
FWVLVVVGGVLACYSLLVTVAFIIFWVHRGRKKLLYIFKQPFMRPVQTTQEEDGCSCRFPEEEEGGCEL

SEQ ID NO: 116 - protein, 69 aa, synthetic construct
  REGION 1..69: note = Synthetic K28L
FWVLVVVGGVLACYSLLVTVAFIIFWVLRGRKKLLYIFKQPFMRPVQTTQEEDGCSCRFPEEEEGGCEL

SEQ ID NO: 117 - protein, 69 aa, synthetic construct
  REGION 1..69: note = Synthetic K28Q
FWVLVVVGGVLACYSLLVTVAFIIFWVQRGRKKLLYIFKQPFMRPVQTTQEEDGCSCRFPEEEEGGCEL

SEQ ID NO: 118 - protein, 69 aa, synthetic construct
  REGION 1..69: note = Synthetic K28S
FWVLVVVGGVLACYSLLVTVAFIIFWVSRGRKKLLYIFKQPFMRPVQTTQEEDGCSCRFPEEEEGGCEL

SEQ ID NO: 119 - protein, 69 aa, synthetic construct
  REGION 1..69: note = Synthetic R31A
FWVLVVVGGVLACYSLLVTVAFIIFWVKRGAKKLLYIFKQPFMRPVQTTQEEDGCSCRFPEEEEGGCEL

SEQ ID NO: 120 - protein, 69 aa, synthetic construct
  REGION 1..69: note = Synthetic R31H
FWVLVVVGGVLACYSLLVTVAFIIFWVKRGHKKLLYIFKQPFMRPVQTTQEEDGCSCRFPEEEEGGCEL

SEQ ID NO: 121 - protein, 69 aa, synthetic construct
  REGION 1..69: note = Synthetic R31L
FWVLVVVGGVLACYSLLVTVAFIIFWVKRGLKKLLYIFKQPFMRPVQTTQEEDGCSCRFPEEEEGGCEL

SEQ ID NO: 122 - protein, 69 aa, synthetic construct
  REGION 1..69: note = Synthetic R31N
FWVLVVVGGVLACYSLLVTVAFIIFWVKRGNKKLLYIFKQPFMRPVQTTQEEDGCSCRFPEEEEGGCEL

SEQ ID NO: 123 - protein, 69 aa, synthetic construct
  REGION 1..69: note = Synthetic L34A
FWVLVVVGGVLACYSLLVTVAFIIFWVKRGRKKALYIFKQPFMRPVQTTQEEDGCSCRFPEEEEGGCEL

SEQ ID NO: 124 - protein, 69 aa, synthetic construct
  REGION 1..69: note = Synthetic L34S
FWVLVVVGGVLACYSLLVTVAFIIFWVKRGRKKSLYIFKQPFMRPVQTTQEEDGCSCRFPEEEEGGCEL

SEQ ID NO: 125 - protein, 69 aa, synthetic construct
  REGION 1..69: note = Synthetic K28Q/R31A
FWVLVVVGGVLACYSLLVTVAFIIFWVQRGAKKLLYIFKQPFMRPVQTTQEEDGCSCRFPEEEEGGCEL

SEQ ID NO: 126 - protein, 69 aa, synthetic construct
  REGION 1..69: note = Synthetic K28Q/R31N
FWVLVVVGGVLACYSLLVTVAFIIFWVQRGNKKLLYIFKQPFMRPVQTTQEEDGCSCRFPEEEEGGCEL

SEQ ID NO: 127 - protein, 69 aa, synthetic construct
  REGION 1..69: note = Synthetic K28Q/R31S
FWVLVVVGGVLACYSLLVTVAFIIFWVQRGSKKLLYIFKQPFMRPVQTTQEEDGCSCRFPEEEEGGCEL

SEQ ID NO: 128 - protein, 69 aa, synthetic construct
  REGION 1..69: note = Synthetic K28Q/L34A
FWVLVVVGGVLACYSLLVTVAFIIFWVQRGRKKALYIFKQPFMRPVQTTQEEDGCSCRFPEEEEGGCEL

SEQ ID NO: 129 - protein, 69 aa, synthetic construct
  REGION 1..69: note = Synthetic K28Q/L34S
FWVLVVVGGVLACYSLLVTVAFIIFWVQRGRKKSLYIFKQPFMRPVQTTQEEDGCSCRFPEEEEGGCEL

SEQ ID NO: 130 - protein, 69 aa, synthetic construct
  REGION 1..69: note = Synthetic R31N/L34A
FWVLVVVGGVLACYSLLVTVAFIIFWVKRGNKKALYIFKQPFMRPVQTTQEEDGCSCRFPEEEEGGCEL

SEQ ID NO: 131 - protein, 69 aa, synthetic construct
  REGION 1..69: note = Synthetic R31N/L34S
FWVLVVVGGVLACYSLLVTVAFIIFWVKRGNKKSLYIFKQPFMRPVQTTQEEDGCSCRFPEEEEGGCEL

SEQ ID NO: 132 - protein, 69 aa, synthetic construct
  REGION 1..69: note = Synthetic K28Q/R31N/L34A
FWVLVVVGGVLACYSLLVTVAFIIFWVQRGNKKALYIFKQPFMRPVQTTQEEDGCSCRFPEEEEGGCEL

SEQ ID NO: 133 - protein, 69 aa, synthetic construct
  REGION 1..69: note = Synthetic K28Q/R31N/L34S
FWVLVVVGGVLACYSLLVTVAFIIFWVQRGNKKSLYIFKQPFMRPVQTTQEEDGCSCRFPEEEEGGCEL

SEQ ID NO: 134 - protein, 71 aa, synthetic construct
  REGION 1..71: note = NN Insertion
FWVLVVVGGVLACYSLLVTVAFIIFWVNNKRGRKKLLYIFKQPFMRPVQTTQEEDGCSCRFPEEEEGGCEL

SEQ ID NO: 135 - protein, 70 aa, synthetic construct
MFWVLVVVGGVLACYSLLVTVAFIIFWVKRGRKKLLYIFKQPFMRPVQTTQEEDGCSCRFPEEEEGGCEL

SEQ ID NO: 136 - protein, 108 aa, synthetic construct
IEVMYPPPYLDNEKSNGTIIHVKGKHLCPSPLFPGPSKPFWVLVVVGGVLACYSLLVTVAFIIFWVKRGRKKLLYIFKQPFMRPVQTTQEEDGCSCRFPEEEEGGCEL

SEQ ID NO: 137 - protein, 26 aa, synthetic construct
  REGION 1..26: note = junction region
SLLVTVAFIIFWVKRGRKKLLYIFKQ

SEQ ID NO: 138 - protein, 26 aa, synthetic construct
  REGION 1..26: note = junction region K14A
SLLVTVAFIIFWVARGRKKLLYIFKQ

SEQ ID NO: 139 - protein, 26 aa, synthetic construct
  REGION 1..26: note = junction region K14H
SLLVTVAFIIFWVHRGRKKLLYIFKQ

SEQ ID NO: 140 - protein, 26 aa, synthetic construct
  REGION 1..26: note = junction region K14L
SLLVTVAFIIFWVLRGRKKLLYIFKQ

SEQ ID NO: 141 - protein, 26 aa, synthetic construct
  REGION 1..26: note = junction region K14Q
SLLVTVAFIIFWVQRGRKKLLYIFKQ

SEQ ID NO: 142 - protein, 26 aa, synthetic construct
  REGION 1..26: note = junction region K14S
SLLVTVAFIIFWVSRGRKKLLYIFKQ

SEQ ID NO: 143 - protein, 26 aa, synthetic construct
  REGION 1..26: note = junction region R17A
SLLVTVAFIIFWVKRGAKKLLYIFKQ

SEQ ID NO: 144 - protein, 26 aa, synthetic construct
  REGION 1..26: note = junction region R17H
SLLVTVAFIIFWVKRGHKKLLYIFKQ

SEQ ID NO: 145 - protein, 26 aa, synthetic construct
  REGION 1..26: note = junction region R17L
SLLVTVAFIIFWVKRGLKKLLYIFKQ

SEQ ID NO: 146 - protein, 26 aa, synthetic construct
  REGION 1..26: note = junction region R17N
SLLVTVAFIIFWVKRGNKKLLYIFKQ

SEQ ID NO: 147 - protein, 26 aa, synthetic construct
  REGION 1..26: note = junction region L20A
SLLVTVAFIIFWVKRGRKKALYIFKQ

SEQ ID NO: 148 - protein, 26 aa, synthetic construct
  REGION 1..26: note = junction region L20S
SLLVTVAFIIFWVKRGRKKSLYIFKQ

SEQ ID NO: 149 - protein, 26 aa, synthetic construct
  REGION 1..26: note = junction region K14Q/R17A
SLLVTVAFIIFWVQRGAKKLLYIFKQ

SEQ ID NO: 150 - protein, 26 aa, synthetic construct
  REGION 1..26: note = junction region K14Q/R17N
SLLVTVAFIIFWVQRGNKKLLYIFKQ

SEQ ID NO: 151 - protein, 26 aa, synthetic construct
  REGION 1..26: note = junction region K14Q/R17S
SLLVTVAFIIFWVQRGSKKLLYIFKQ

SEQ ID NO: 152 - protein, 26 aa, synthetic construct
  REGION 1..26: note = junction region K14Q/L20A
SLLVTVAFIIFWVQRGRKKALYIFKQ

SEQ ID NO: 153 - protein, 26 aa, synthetic construct
  REGION 1..26: note = junction region K14Q/L20S
SLLVTVAFIIFWVQRGRKKSLYIFKQ

SEQ ID NO: 154 - protein, 26 aa, synthetic construct
  REGION 1..26: note = junction region R17N/L20A
SLLVTVAFIIFWVKRGNKKALYIFKQ

SEQ ID NO: 155 - protein, 26 aa, synthetic construct
  REGION 1..26: note = junction region R17N/L20S
SLLVTVAFIIFWVKRGNKKSLYIFKQ

SEQ ID NO: 156 - protein, 26 aa, synthetic construct
  REGION 1..26: note = junction region K14Q/R17N/L20A
SLLVTVAFIIFWVQRGNKKALYIFKQ

SEQ ID NO: 157 - protein, 26 aa, synthetic construct
  REGION 1..26: note = junction region K14Q/R17N/L20S
SLLVTVAFIIFWVQRGNKKSLYIFKQ

SEQ ID NO: 158 - DNA, 36 bp, Homo sapiens; identical to SEQ ID NO: 106
  misc_feature 1..36: note = spacer (IgG4hinge)
  source 1..36: mol_type = unassigned DNA

SEQ ID NO: 159 - protein, 112 aa, synthetic construct
  REGION 1..112: note = CD3 Zeta
RVKFSRSADAPAYKQGQNQLYNELNLGRREEYDVLDKRRGRDPEMGGKPRRKNPQEGLYNELQKDKMAEAYSEIGMKGERRRGKGHDGLYQGLSTATKDTYDALHMQALPPR

SEQ ID NO: 160 - protein, 36 aa, synthetic construct
CYSLLVTVAFIIFWVKRGRKKLLYIFKQPFMRPVQT

SEQ ID NO: 161 - protein, 15 aa, synthetic construct
CYSLLVTVAFIIFWV

SEQ ID NO: 162 - protein, 15 aa, synthetic construct
LLVTVAFIIFWVKRG

SEQ ID NO: 163 - protein, 15 aa, synthetic construct
TVAFIIFWVKRGRKK

SEQ ID NO: 164 - protein, 15 aa, synthetic construct
FIIFWVKRGRKKLLY

SEQ ID NO: 165 - protein, 15 aa, synthetic construct
FWVKRGRKKLLYIFK

SEQ ID NO: 166 - protein, 15 aa, synthetic construct
KRGRKKLLYIFKQPF

SEQ ID NO: 167 - protein, 15 aa, synthetic construct
RKKLLYIFKQPFMRP

SEQ ID NO: 168 - protein, 15 aa, synthetic construct
LLYIFKQPFMRPVQT

SEQ ID NO: 169 - protein, 15 aa, synthetic construct
  REGION 1..15: note = Synthetic peptide R31H
TVAFIIFWVKRGHKK

SEQ ID NO: 170 - protein, 15 aa, synthetic construct
  REGION 1..15: note = Synthetic peptide R31H
FIIFWVKRGHKKLLY

SEQ ID NO: 171 - protein, 15 aa, synthetic construct
  REGION 1..15: note = Synthetic peptide R31H
FWVKRGHKKLLYIFK

SEQ ID NO: 172 - protein, 15 aa, synthetic construct
  REGION 1..15: note = Synthetic peptide R31H
KRGHKKLLYIFKQPF

SEQ ID NO: 173 - protein, 15 aa, synthetic construct
  REGION 1..15: note = Synthetic peptide R31H
HKKLLYIFKQPFMRP

SEQ ID NO: 174 - protein, 15 aa, synthetic construct
  REGION 1..15: note = Synthetic peptide R31N
TVAFIIFWVKRGNKK

SEQ ID NO: 175 - protein, 15 aa, synthetic construct
  REGION 1..15: note = Synthetic peptide R31N
FIIFWVKRGNKKLLY

SEQ ID NO: 176 - protein, 15 aa, synthetic construct
  REGION 1..15: note = Synthetic peptide R31N
FWVKRGNKKLLYIFK

SEQ ID NO: 177 - protein, 15 aa, synthetic construct
  REGION 1..15: note = Synthetic peptide R31N
KRGNKKLLYIFKQPF

SEQ ID NO: 178 - protein, 15 aa, synthetic construct
  REGION 1..15: note = Synthetic peptide R31N
NKKLLYIFKQPFMRP

SEQ ID NO: 179 - protein, 15 aa, synthetic construct
  REGION 1..15: note = Synthetic peptide L34A
FIIFWVKRGRKKALY

SEQ ID NO: 180 - protein, 15 aa, synthetic construct
  REGION 1..15: note = Synthetic peptide L34A
FWVKRGRKKALYIFK

SEQ ID NO: 181 - protein, 15 aa, synthetic construct
  REGION 1..15: note = Synthetic peptide L34A
KRGRKKALYIFKQPF

SEQ ID NO: 182 - protein, 15 aa, synthetic construct
  REGION 1..15: note = Synthetic peptide L34A
RKKALYIFKQPFMRP

SEQ ID NO: 183 - protein, 69 aa, synthetic construct
  REGION 1..69: note = Synthetic R31S
FWVLVVVGGVLACYSLLVTVAFIIFWVKRGSKKLLYIFKQPFMRPVQTTQEEDGCSCRFPEEEEGGCEL

SEQ ID NO: 184 - protein, 26 aa, synthetic construct
  REGION 1..26: note = junction region R31S
SLLVTVAFIIFWVKRGSKKLLYIFKQ